European Patent Specification EP 3 854 880 B1, published July 17, 2024. Title: Method for screening for proteins protecting client proteins. Applicant: The University of Tokyo. The sequence listing filed with the application follows.

SEQUENCE LISTING (40 sequences)

SEQ ID NO: 1 - protein, 59 aa, Homo sapiens
MTRGNQRELARQKNMKKQSDSVKGKRRDDGLSAAARKQRDSEIMQQKQKKANEKKEEPK

SEQ ID NO: 2 - protein, 83 aa, Homo sapiens
MSGPNGDLGMPVEAGAEGEEDGFGEAEYAAINSMLDQINSCLDHLEEKNDHLHARLQELLESNRQTRLEFQQQLGEAPSDASP

SEQ ID NO: 3 - protein, 99 aa, Homo sapiens
MAQGQRKFQAHKPAKSKTAAAASEKNRGPRKGGRVIAPKKARVVQQQKLKKNLEVGIRKKIEHDVVMKASSSLPKKLALLKAPAKKKGAAAATSSKTPS

SEQ ID NO: 4 - protein, 111 aa, Homo sapiens
MANIHQENEEMEQPMQNGEEDRPLGGGEGHQPAGNRRGQARRLAPNFRWAIPNRQINDGMGGDGDDMEIFMEEMREIRRKLRELQLRNCLRILMGELSNHHDHHDEFCLMP

SEQ ID NO: 5 - protein, 182 aa, Homo sapiens
MSAARESHPHGVKRSASPDDDLGSSNWEAADLGNEERKQKFLRLMGAGKKEHTGRLVIGDHKSTSHFRTGEEDKKINEELESQYQQSMDSKLSGRYRRHCGLGFSEVEDHDGEGDVAGDDDDDDDDSPDPESPDDSESDSESEKEESAEELQAAEHPDEVEDPKNKKDAKSNYKMMFVKSSG

SEQ ID NO: 6 - protein, 408 aa, Homo sapiens
MPGHLQEGFGCVVTNRFDQLFDDESDPFEVLKAAENKKKEAGGGGVGGPGAKSAAQAAAQTNSNAAGKQLRKESQKDRKNPLPPSVGVVDKKEETQPPVALKKEGIRRVGRRPDQQLQGEGKIIDRRPERRPPRERRFEKPLEEKGEGGEFSVDRPIIDRPIRGRGGLGRGRGGRGRGMGRGDGFDSRGKREFDRHSGSDRSSFSHYSGLKHEDKRGGSGSHNWGTVKDELTESPKYIQKQISYNYSDLDQSNVTEETPEGEEHHPVADTENKENEVEEVKEEGPKEMTLDEWKAIQNKDRAKVEFNIRKPNEGADGQWKKGFVLHKSKSEEAHAEDSVMDHHFRKPANDITSQLEINFGDLGRPGRGGRGGRGGRGRGGRPNRGSRTDKSSASAPDVDDPEAFPALA

SEQ ID NO: 7 - protein, 118 aa, Drosophila melanogaster
MTSTELKIGLTTSARPSSRVLKPPGGGHTNIFSEPDVAVPAPRAKYNQQNSSNLNACMGSTDPNKVVEKIREEVSIQKEEAKSAPPSQPKEPANKPAATNGEARGRVPPGGFSSGGFW

SEQ ID NO: 8 - protein, 61 aa, Drosophila melanogaster
MTSTELKIGLTTSARPSSRVLKPPGGGHTNIFSEPDVAVPAPRAKYNQQNSSNLNACMGST

SEQ ID NO: 9 - protein, 57 aa, Drosophila melanogaster
DPNKVVEKIREEVSIQKEEAKSAPPSQPKEPANKPAATNGEARGRVPPGGFSSGGFW

SEQ ID NO: 10 - protein, 96 aa, Drosophila melanogaster
MADEQPNLVAGHPPALKAGGMRIVQHKAPTAERAPKDAEDCTGLTQPIAVNSGSVSGAPVKGNTDFTPASAQVAHSPKPPAAVQQKPQIHIQQPRK

SEQ ID NO: 11 - protein, 48 aa, Drosophila melanogaster
MADEQPNLVAGHPPALKAGGMRIVQHKAPTAERAPKDAEDCTGLTQPI

SEQ ID NO: 12 - protein, 48 aa, Drosophila melanogaster
AVNSGSVSGAPVKGNTDFTPASAQVAHSPKPPAAVQQKPQIHIQQPRK

SEQ ID NO: 13 - protein, 96 aa, Drosophila melanogaster
MSPKNNHDPSSSGDSGNTNVQEADLQEMEDVNNSLDALSCALDAVEQRTDDIMSQLRELLNSNREIRRLIAEENDNAPESGDDNMDGQAGSEAAPK

SEQ ID NO: 14 - protein, 48 aa, Drosophila melanogaster
MSPKNNHDPSSSGDSGNTNVQEADLQEMEDVNNSLDALSCALDAVEQR

SEQ ID NO: 15 - protein, 48 aa, Drosophila melanogaster
TDDIMSQLRELLNSNREIRRLIAEENDNAPESGDDNMDGQAGSEAAPK

SEQ ID NO: 16 - protein, 41 aa, Homo sapiens
MSGPNGDLGMPVEAGAEGEEDGFGEAEYAAINSMLDQINSC

SEQ ID NO: 17 - protein, 42 aa, Homo sapiens
LDHLEEKNDHLHARLQELLESNRQTRLEFQQQLGEAPSDASP

SEQ ID NO: 18 - protein, 60 aa, Homo sapiens
MSAARESHPHGVKRSASPDDDLGSSNWEAADLGNEERKQKFLRLMGAGKKEHTGRLVIGD

SEQ ID NO: 19 - protein, 98 aa, Homo sapiens
QSMDSKLSGRYRRHCGLGFSEVEDHDGEGDVAGDDDDDDDDSPDPESPDDSESDSESEKEESAEELQAAEHPDEVEDPKNKKDAKSNYKMMFVKSSGS

SEQ ID NO: 20 - protein, 100 aa, Homo sapiens
QAKARSAAKGEMEQAKRNQIKSEQRAEKKSMNQQRKTQGLQNDEGRSSRDARIKLQPKKVMDKQGDDKKDQKEKDTRSKRPGLRKKRNVQRENEKSKAMM

SEQ ID NO: 21 - protein, 100 aa, Homo sapiens
KKNDKSKRDKQVRKSAKIKQGQNRMQKAQLNKQMSTKSRQQQLREDPKEGRQGREADSGEKEKAPERRKSKDKADQRMNTAELKSGARRVKKADEIMMQN

SEQ ID NO: 22 - protein, 100 aa, Homo sapiens
QKMVKKQGQIKKDKKDRQAKENQNKELAKQRRGVSEKEMDTILAQEDMSPAAKRDKEMDGMQSKRNSKSKRKRQARGEKQTDPGLRRKSKSARQARENQN

SEQ ID NO: 23 - protein, 42 aa, Homo sapiens
QSDEPMIVRQAQRKMDQRKKKGLEKKADAKKNGNERSQRSAT

SEQ ID NO: 24 - protein, 42 aa, Homo sapiens
RKQDKNGRKSEKLNAMGQAADMKSERERVISPTQQQKKADKR

SEQ ID NO: 25 - protein, 100 aa, Homo sapiens
GKPKQAKLSEKSSFQAPAVGPLVKRRENARRAKAVTKLQEKKHIAKTVMKSVKKKLIASKNTASMSKRAQASPKQGLVKGQHARAPKAIKAALKGGPAKD

SEQ ID NO: 26 - protein, 100 aa, Homo sapiens
SAPSKVKQRIVPKNKSAAKKPFSSDAVKRKSQKERAEMTGVKEGAKLKKALAAKPLIKPAPMKKATAAKNRAHIAVKVKAKHGSGQGQTLQKLRLGSRAQ

SEQ ID NO: 27 - protein, 100 aa, Homo sapiens
QMSPKQKRTSAKVKAVGILAKLKPSASQLAHNSAKKAEKRVPLIKVTIGPQLAGKAQSDVNMLRSAKGAKKVKEKPFKARGAKSKQTAHPRKAKEGRKAA

SEQ ID NO: 28 - protein, 42 aa, Homo sapiens
RAKKPKQKHKKAGRKGGAAMAVSPLLPVAVLNSRQESKKIAT

SEQ ID NO: 29 - protein, 42 aa, Homo sapiens
GKKHRRTANAAAAVKQAQGVKKPPKSKGLLMPLQKIRSASEK

SEQ ID NO: 30 - protein, 100 aa, Homo sapiens
RRQAGVGKIRMDTGPAANGSRDNGKKVKVKDSLASFKNAREEPGFPQDLTKSKYHEIRGGDEERDRPPRGIDGPSHGVEGLHGNFEQVESWRSLAEQGTE

SEQ ID NO: 31 - protein, 100 aa, Homo sapiens
RPKLEQVGLAEPFRSPGKTRSEHTNHEDNGEERLMGAVGKGGQGDFRHSATVADRGIGVEFRESANKYKKEPLGKIQVQGDWNSDARGDPDGRESSKPRI

SEQ ID NO: 32 - protein, 100 aa, Homo sapiens
QNANQGARPFAGFLAVPDKEQREKDIFEQGPERLLGSPDGGGSGYRGRIKKMVRDHPGKSSHSDAKEKSRRGVTPWDEDRSVEEGAERGVNTILGTEHNK

SEQ ID NO: 33 - protein, 42 aa, Homo sapiens
QGDRRKLSNGENDQAEDETKFPGHGPRKPAIGAKESSRGVVL

SEQ ID NO: 34 - protein, 42 aa, Homo sapiens
PRRAKIEHQLAKDNDRGSGGGVANRKPEEQGSGPKDVETSLF

SEQ ID NO: 35 - protein, 218 aa, Homo sapiens
MSPILGYWKIKGLVQPTRLLLEYLEEKYEEHLYERDEGDKWRNKKFELGLEFPNLPYYIDGDVKLTQSMAIIRYIADKHNMLGGCPKERAEISMLEGAVLDIRYGVSRIAYSKDFETLKVDFLSKLPEMLKMFEDRLCHKTYLNGDHVTHPDFMLYDALDVVLYMDPMCLDAFPKLVCFKKRIEAIPQIDKYLKSSKYIAWPLQGWQATFGGGDHPPK

SEQ ID NO: 36 - protein, 100 aa, Homo sapiens
DIISKTKEAIVPEKYHMPAKRGQETPVLNYYLLIASLTNIKDFMDKGDPLIFDPFKQYSSAKRDLKADHGLFLKLPVECGWYVRCGLLRYLEMGHMEEWD

SEQ ID NO: 37 - protein, 100 aa, Homo sapiens
CRPAIVMHGVEKTEDMKIWLLWKKSKLNPIENEKALQVLPDPRDALRLCPELDHGMFDKMVPSDAGGIKYAFYYEGSHGKYLFSIFLQTRLDKIETDYLY

SEQ ID NO: 38 - protein, 100 aa, Homo sapiens
CDAKFLGILLLKLKKYKHIQDHDFRIKHIDVLGPVPGLMYAESDCIYTPAEIATYDEYFKREEPYMWKELVWESGLDDLSMANTGFSRPMPNLKLQVKGR

SEQ ID NO: 39 - protein, 42 aa, Homo sapiens
HLEFVNFVPIGPCGDLYRLEEQKLAYKDMMIRSDAYKGKWTL

SEQ ID NO: 40 - protein, 42 aa, Homo sapiens
FESFYMEPLLWTDKINHLYYLIGAKDPVLGKRDVKREQAMGC